European Patent Application EP 4 140 501 A1, published March 1, 2023. Title: Improved peptide vaccines. Applicant: BrightPath Biotherapeutics Co., Ltd. Kagoshima University. The sequence listing filed with the application follows.

SEQUENCE LISTING (103 sequences)

SEQ ID NO: 1 - protein, 17 aa, Artificial Sequence
  Type 1 IgG binding peptide
  MISC_FEATURE (1)..(1): Xaa can be any naturally occurring amino acid other than Cys or null, or can be Arg-Arg-Gly-Pro together with Xaa at position (2).
  MISC_FEATURE (2)..(2): Xaa can be any naturally occurring amino acid other than Cys or null, or can be Arg-Arg-Gly-Pro together with Xaa at position (1).
  MISC_FEATURE (3)..(3): Xaa can be naturally occurring amino acid other than Cys.
  MISC_FEATURE (5)..(5): Xaa can be naturally occurring amino acid other than Cys.
  MISC_FEATURE (6)..(6): Xaa can be naturally occurring amino acid other than Cys.
  MISC_FEATURE (8)..(8): Xaa is selected from the group consisting of Lys, Cys, Asp, Glu, Arg, Leu, 2-aminosuberic acid, or diaminopropionic acid.
  MISC_FEATURE (10)..(10): Xaa is Glu, Asn or Gln
  MISC_FEATURE (15)..(15): Xaa can be naturally occurring amino acid other than Cys.
  MISC_FEATURE (16)..(16): Xaa can be any naturally occurring amino acid other than Cys or null.
  MISC_FEATURE (17)..(17): Xaa can be any naturally occurring amino acid other than Cys or null.
XXXCXXHXGXLVWCXXX

SEQ ID NO: 2 - protein, 35 aa, Artificial Sequence
  Type 2 IgG binding peptide
  MISC_FEATURE (1)..(1): Xaa is selected from the group consisting of Gly, Ala, Val, Leu, Ile, Met, Pro, Phe, Trp, Lys, ornithine, Cys, Aso, Glu, beta-Ala, 2-aminosuberic acid, diaminopropionic acid, and NH 2-(PEG)n-CO (n=1 `50), or null.
  MISC_FEATURE (2)..(2): Xaa is selected from the group consisting of Lys, ornithine, Cys, Asp, Glu, Phe, 2-aminosuberic acid, and diaminopropionic acid, or null.
  MISC_FEATURE (27)..(27): Xaa is selected from the group consisting of Arg, His, Asp, Glu, Ser, Thr, Asn, Gln, Tyr, and Cys.
  MISC_FEATURE (29)..(29): Xaa is selected from the group consisting of Arg, His, Asp, Glu, Ser, Thr, Asn, Gln, Tyr, and Cys, or null.
XXNMQCQRRFYEALHDPNLNEEQRNAXIXSIRDDC

SEQ ID NO: 3 - protein, 13 aa, Artificial Sequence
  Specific sequence of Type 1 IgG binding peptide.
  MISC_FEATURE (6)..(6): Xaa is selected from the group consisting of Lys, Cys, Asp, Glu, Arg, Leu, 2-aminosuberic acid, or diaminopropionic acid.
DCAYHXGELVWCT

SEQ ID NO: 4 - protein, 17 aa, Artificial Sequence
  Specific sequence of Type 1 IgG binding peptide.
  MISC_FEATURE (8)..(8): Xaa is selected from the group consisting of Lys, Cys, Asp, Glu, Arg, Leu, 2-aminosuberic acid, or diaminopropionic acid.
GPDCAYHXGELVWCTFH

SEQ ID NO: 5 - protein, 13 aa, Artificial Sequence
  Specific sequence of Type 1 IgG binding peptide.
  MISC_FEATURE (6)..(6): Xaa is selected from the group consisting of Lys, Cys, Asp, Glu, Arg, Leu, 2-aminosuberic acid, or diaminopropionic acid.
RCAYHXGELVWCS

SEQ ID NO: 6 - protein, 17 aa, Artificial Sequence
  Specific sequence of Type 1 IgG binding peptide.
  MISC_FEATURE (8)..(8): Xaa is selected from the group consisting of Lys, Cys, Asp, Glu, Arg, Leu, 2-aminosuberic acid, or diaminopropionic acid.
GPRCAYHXGELVWCSFH

SEQ ID NO: 7 - protein, 17 aa, Artificial Sequence
  Specific sequence of Type 1 IgG binding peptide.
  MISC_FEATURE (8)..(8): Xaa is selected from the group consisting of Lys, Cys, Asp, Glu, Arg, Leu, 2-aminosuberic acid, or diaminopropionic acid.
SPDCAYHXGELVWCTFH

SEQ ID NO: 8 - protein, 17 aa, Artificial Sequence
  Specific sequence of Type 1 IgG binding peptide.
  MISC_FEATURE (8)..(8): Xaa is selected from the group consisting of Lys, Cys, Asp, Glu, Arg, Leu, 2-aminosuberic acid, or diaminopropionic acid.
GDDCAYHXGELVWCTFH

SEQ ID NO: 9 - protein, 17 aa, Artificial Sequence
  Specific sequence of Type 1 IgG binding peptide.
  MISC_FEATURE (8)..(8): Xaa is selected from the group consisting of Lys, Cys, Asp, Glu, Arg, Leu, 2-aminosuberic acid, or diaminopropionic acid.
GPSCAYHXGELVWCTFH

SEQ ID NO: 10 - protein, 17 aa, Artificial Sequence
  Specific sequence of Type 1 IgG binding peptide.
  MISC_FEATURE (8)..(8): Xaa is selected from the group consisting of Lys, Cys, Asp, Glu, Arg, Leu, 2-aminosuberic acid, or diaminopropionic acid.
GPDCAYHXGELVWCSFH

SEQ ID NO: 11 - protein, 17 aa, Artificial Sequence
  Specific sequence of Type 1 IgG binding peptide.
  MISC_FEATURE (8)..(8): Xaa is selected from the group consisting of Lys, Cys, Asp, Glu, Arg, Leu, 2-aminosuberic acid, or diaminopropionic acid.
GPDCAYHXGELVWCTHH

SEQ ID NO: 12 - protein, 17 aa, Artificial Sequence
  Specific sequence of Type 1 IgG binding peptide.
  MISC_FEATURE (8)..(8): Xaa is selected from the group consisting of Lys, Cys, Asp, Glu, Arg, Leu, 2-aminosuberic acid, or diaminopropionic acid.
GPDCAYHXGELVWCTFY

SEQ ID NO: 13 - protein, 17 aa, Artificial Sequence
  Specific sequence of Type 1 IgG binding peptide.
  MISC_FEATURE (8)..(8): Xaa is selected from the group consisting of Lys, Cys, Asp, Glu, Arg, Leu, 2-aminosuberic acid, or diaminopropionic acid.
SPDCAYHXGELVWCTFY

SEQ ID NO: 14 - protein, 17 aa, Artificial Sequence
  Specific sequence of Type 1 IgG binding peptide.
  MISC_FEATURE (8)..(8): Xaa is selected from the group consisting of Lys, Cys, Asp, Glu, Arg, Leu, 2-aminosuberic acid, or diaminopropionic acid.
SDDCAYHXGELVWCTFY

SEQ ID NO: 15 - protein, 17 aa, Artificial Sequence
  Specific sequence of Type 1 IgG binding peptide.
  MISC_FEATURE (8)..(8): Xaa is selected from the group consisting of Lys, Cys, Asp, Glu, Arg, Leu, 2-aminosuberic acid, or diaminopropionic acid.
RGNCAYHXGQLVWCTYH

SEQ ID NO: 16 - protein, 17 aa, Artificial Sequence
  Specific sequence of Type 1 IgG binding peptide.
  MISC_FEATURE (2)..(2): Xaa can be any naturally occurring amino acid other than Cys or null.
  MISC_FEATURE (8)..(8): Xaa is selected from the group consisting of Lys, Cys, Asp, Glu, Arg, Leu, 2-aminosuberic acid, or diaminopropionic acid.
  MISC_FEATURE (16)..(16): Xaa can be any naturally occurring amino acid other than Cys or null.
GXDCAYHXGELVWCTXH

SEQ ID NO: 17 - protein, 19 aa, Artificial Sequence
  Specific sequence of Type 1 IgG binding peptide.
  MISC_FEATURE (10)..(10): Xaa is selected from the group consisting of Lys, Cys, Asp, Glu, Arg, Leu, 2-aminosuberic acid, or diaminopropionic acid.
RRGPDCAYHXGELVWCTFH

SEQ ID NO: 18 - protein, 34 aa, Artificial Sequence
  Specific sequence of Type 2 IgG binding peptide.
FNMQCQRRFYEALHDPNLNEEQRNARIRSIRDDC

SEQ ID NO: 19 - protein, 35 aa, Artificial Sequence
  Specific sequence of Type 2 IgG binding peptide.
GFNMQCQRRFYEALHDPNLNEEQRNARIRSIRDDC

SEQ ID NO: 20 - protein, 34 aa, Artificial Sequence
  Specific sequence of Type 2 IgG binding peptide.
KNMQCQRRFYEALHDPNLNEEQRNARIRSIRDDC

SEQ ID NO: 21 - protein, 35 aa, Artificial Sequence
  Specific sequence of Type 2 IgG binding peptide.
GFNMQCQKRFYEALHDPNLNEEQRNARIRSIRDDC

SEQ ID NO: 22 - protein, 34 aa, Artificial Sequence
  Specific sequence of Type 2 IgG binding peptide.
KNMQCQKRFYEALHDPNLNEEQRNARIRSIRDDC

SEQ ID NO: 23 - protein, 33 aa, Artificial Sequence
  Specific sequence of Type 2 IgG binding peptide.
FNMQQQRRFYEALHDPNLNEEQRNARIRSIRDD

SEQ ID NO: 24 - protein, 35 aa, Artificial Sequence
  Specific sequence of Type 2 IgG binding peptide.
GKNMQCQRRFYEALHDPNLNEEQRNARIRSIRDDC

SEQ ID NO: 25 - protein, 17 aa, Artificial Sequence
  IgG Binding Peptide (1)
GPDCAYHRGELVWCTFH

SEQ ID NO: 26 - protein, 17 aa, Artificial Sequence
  IgG Binding Peptide (2)
GPDCAYHKGELVWCTFH

SEQ ID NO: 27 - protein, 17 aa, Artificial Sequence
  IgG Binding Peptide (Negative Control)
GPDCAYHRGEAAACTFH

SEQ ID NO: 28 - protein, 8 aa, Artificial Sequence
  Amino acid sequence of antigen Peptide (1) derived from OVA.
SIINFEKL

SEQ ID NO: 29 - protein, 16 aa, Artificial Sequence
  Amino acid sequence of antigen Peptide (2) derived from OVA.
EQLESIINFEKLTEWT

SEQ ID NO: 30 - protein, 33 aa, Artificial Sequence
  Amino acid sequence of Peptide (3-1) generated from Peptide (2) linked with IgG BP(1).
EQLESIINFEKLTEWTGPDCAYHRGELVWCTFH

SEQ ID NO: 31 - protein, 33 aa, Artificial Sequence
  Amino acid sequence of Peptide (4) generated from Peptide (2) linked with IgG BP(NC).
EQLESIINFEKLTEWTGPDCAYHRGEAAACTFH

SEQ ID NO: 32 - protein, 8 aa, Artificial Sequence
  Amino acid sequence of antigenic Peptide (5) derived from CMV.
PVAALFFF

SEQ ID NO: 33 - protein, 16 aa, Artificial Sequence
  Amino acid sequence of Peptide (6) derived from CMV.
RQYDPVAALFFFDIDL

SEQ ID NO: 34 - protein, 33 aa, Artificial Sequence
  Amino acid sequence of Peptide (7) generated from Peptide (6) linked with IgG BP(2).
RQYDPVAALFFFDIDLGPDCAYHKGELVWCTFH

SEQ ID NO: 35 - protein, 9 aa, Artificial Sequence
  Amino acid sequence of Peptide (8) derived from neoantigen Adpgk.
ASMTNMELM

SEQ ID NO: 36 - protein, 17 aa, Artificial Sequence
  Amino acid sequence of Peptide (9) derived from neoantigen Adpgk.
HLELASMTNMELMSSIV

SEQ ID NO: 37 - protein, 34 aa, Artificial Sequence
  Amino acid sequence of Peptide (10) generated from Peptide (9) linked with IgG BP(1).
HLELASMTNMELMSSIVGPDCAYHRGELVWCTFH

SEQ ID NO: 38 - protein, 34 aa, Artificial Sequence
  Amino acid sequence of Peptide (11) generated from Peptide (9) linked with IgG BP(NC).
HLELASMTNMELMSSIVGPDCAYHRGEAAACTFH

SEQ ID NO: 39 - protein, 17 aa, Artificial Sequence
  IgG Binding Peptide (3)
GPDCAWHRGELVWCTFH

SEQ ID NO: 40 - protein, 17 aa, Artificial Sequence
  IgG Binding Peptide (4)
GPDCAWHLGELVWCTFH

SEQ ID NO: 41 - protein, 33 aa, Artificial Sequence
  Amino acid sequence of Peptide (3-2) generated from Peptide (2) linked with IgG BP(2).
EQLESIINFEKLTEWTGPDCAYHKGELVWCTFH

SEQ ID NO: 42 - protein, 33 aa, Artificial Sequence
  Amino acid sequence of Peptide (3-3) generated from Peptide (2) linked with IgG BP(3).
EQLESIINFEKLTEWTGPDCAWHRGELVWCTFH

SEQ ID NO: 43 - protein, 33 aa, Artificial Sequence
  Amino acid sequence of Peptide (3-4) generated from Peptide (2) linked with IgG BP(4).
EQLESIINFEKLTEWTGPDCAWHLGELVWCTFH

SEQ ID NO: 44 - protein, 27 aa, Artificial Sequence
  Amino acid sequence of antigenic Peptide (101) derived from murine cancer cell line.
KLAEGAERDGKNNVAFMSYFLQGTLDA

SEQ ID NO: 45 - protein, 27 aa, Artificial Sequence
  Amino acid sequence of antigenic Peptide (102) derived from murine cancer cell line.
LLQFEVCPLSESRFSLSFQHPVNDSLV

SEQ ID NO: 46 - protein, 27 aa, Artificial Sequence
  Amino acid sequence of antigenic Peptide (103) derived from murine cancer cell line.
TEPIYQPHSAWVPFGGLMGLALLGALL

SEQ ID NO: 47 - protein, 27 aa, Artificial Sequence
  Amino acid sequence of antigenic Peptide (104) derived from murine cancer cell line.
PPRALPPVPSAIQANIPLSHPKKKKSR

SEQ ID NO: 48 - protein, 27 aa, Artificial Sequence
  Amino acid sequence of antigenic Peptide (105) derived from murine cancer cell line.
AHDSSKDSVTVFVNNLPYSIEEPEVKL

SEQ ID NO: 49 - protein, 27 aa, Artificial Sequence
  Amino acid sequence of antigenic Peptide (106) derived from murine cancer cell line.
RTPKLSSIIDCTGTASYNGFLPVLVRN

SEQ ID NO: 50 - protein, 27 aa, Artificial Sequence
  Amino acid sequence of antigenic Peptide (107) derived from murine cancer cell line.
IILGKSHYVLYGLIAAMQPRMLVTFDE

SEQ ID NO: 51 - protein, 27 aa, Artificial Sequence
  Amino acid sequence of antigenic Peptide (108) derived from murine cancer cell line.
HQVRVYDPVSPQHRPVLEATYGEYPLE

SEQ ID NO: 52 - protein, 27 aa, Artificial Sequence
  Amino acid sequence of antigenic Peptide (109) derived from murine cancer cell line.
TSSGPGVTSAVDFKLHIEVLHYLLQSW

SEQ ID NO: 53 - protein, 27 aa, Artificial Sequence
  Amino acid sequence of antigenic Peptide (110) derived from murine cancer cell line.
EASEEGEEEEDEEDLEAMQSRLPTLRS

SEQ ID NO: 54 - protein, 27 aa, Artificial Sequence
  Amino acid sequence of antigenic Peptide (111) derived from murine cancer cell line.
LEIDHYVGSAPPLLEGPLPSRNSVPIL

SEQ ID NO: 55 - protein, 27 aa, Artificial Sequence
  Amino acid sequence of antigenic Peptide (112) derived from murine cancer cell line.
NEQDSLVVLDVTASLKIRNSNFYPVAV

SEQ ID NO: 56 - protein, 27 aa, Artificial Sequence
  Amino acid sequence of antigenic Peptide (113) derived from murine cancer cell line.
GIPVHLELASMTNMELMSSIVHQVFPT

SEQ ID NO: 57 - protein, 27 aa, Artificial Sequence
  Amino acid sequence of antigenic Peptide (114) derived from murine cancer cell line.
LLPTEQRMLMKSVLTRLRTPMNLPKLM

SEQ ID NO: 58 - protein, 27 aa, Artificial Sequence
  Amino acid sequence of antigenic Peptide (115) derived from murine cancer cell line.
MTPELQEKMVSFRSIFKDLEDKKVNQQ

SEQ ID NO: 59 - protein, 27 aa, Artificial Sequence
  Amino acid sequence of antigenic Peptide (116) derived from murine cancer cell line.
TRTSSSSLTSSVPVAPQLEEAPLTVKS

SEQ ID NO: 60 - protein, 27 aa, Artificial Sequence
  Amino acid sequence of antigenic Peptide (117) derived from murine cancer cell line.
GPDIHRIQEKPRNNRVAVATINFRRLV

SEQ ID NO: 61 - protein, 27 aa, Artificial Sequence
  Amino acid sequence of antigenic Peptide (118) derived from murine cancer cell line.
DDDETGKISFKNLTRVAKELGENLTDE

SEQ ID NO: 62 - protein, 27 aa, Artificial Sequence
  Amino acid sequence of antigenic Peptide (119) derived from murine cancer cell line.
HESGHAIIAYYTKAAMPINKATIMPRG

SEQ ID NO: 63 - protein, 27 aa, Artificial Sequence
  Amino acid sequence of antigenic Peptide (120) derived from murine cancer cell line.
KRNENCTLQFEAALALTNIASGTSQQT

SEQ ID NO: 64 - protein, 27 aa, Artificial Sequence
  Amino acid sequence of antigenic Peptide (121) derived from murine cancer cell line.
EALAQKTYSDDHVTFFCFQVLEHQVKY

SEQ ID NO: 65 - protein, 27 aa, Artificial Sequence
  Amino acid sequence of antigenic Peptide (122) derived from murine cancer cell line.
GHGHWVNTMALSTYYALRTGAFEPAEA

SEQ ID NO: 66 - protein, 27 aa, Artificial Sequence
  Amino acid sequence of antigenic Peptide (123) derived from murine cancer cell line.
YPFYSFCDVKQYIEHSILRVAETGPEH

SEQ ID NO: 67 - protein, 27 aa, Artificial Sequence
  Amino acid sequence of antigenic Peptide (124) derived from murine cancer cell line.
AKMKGYPHWPALIDDIADGAVKPPPID

SEQ ID NO: 68 - protein, 27 aa, Artificial Sequence
  Amino acid sequence of antigenic Peptide (125) derived from murine cancer cell line.
NSRLTADLSAQLQNLTSTESQLKEVRS

SEQ ID NO: 69 - protein, 27 aa, Artificial Sequence
  Amino acid sequence of antigenic Peptide (126) derived from murine cancer cell line.
EVGCRGPEASPVSPGEPLRRASRSGGR

SEQ ID NO: 70 - protein, 27 aa, Artificial Sequence
  Amino acid sequence of antigenic Peptide (127) derived from murine cancer cell line.
WTVTLYPSSPVTNYRWRSFTGAVTLEK

SEQ ID NO: 71 - protein, 27 aa, Artificial Sequence
  Amino acid sequence of antigenic Peptide (128) derived from murine cancer cell line.
ASSLIAHVRQHTGRSPTSVNAVARDLS

SEQ ID NO: 72 - protein, 27 aa, Artificial Sequence
  Amino acid sequence of antigenic Peptide (129) derived from murine cancer cell line.
LWISTRIWALWSWVSWNQDPFLKASSL

SEQ ID NO: 73 - protein, 27 aa, Artificial Sequence
  Amino acid sequence of antigenic Peptide (130) derived from murine cancer cell line.
RDGFLGPPNPPFLWALRIRITLPFPQP

SEQ ID NO: 74 - protein, 9 aa, Artificial Sequence
  Amino acid sequence of epitope Peptide (101e) derived from murine cancer cell line.
MSYFLQGTL

SEQ ID NO: 75 - protein, 9 aa, Artificial Sequence
  Amino acid sequence of epitope Peptide (102e) derived from murine cancer cell line.
FSLSFQHPV

SEQ ID NO: 76 - protein, 9 aa, Artificial Sequence
  Amino acid sequence of epitope Peptide (103e) derived from murine cancer cell line.
SAWVPFGGL

SEQ ID NO: 77 - protein, 9 aa, Artificial Sequence
  Amino acid sequence of epitope Peptide (104e) derived from murine cancer cell line.
SAIQANIPL

SEQ ID NO: 78 - protein, 9 aa, Artificial Sequence
  Amino acid sequence of epitope Peptide (105e) derived from murine cancer cell line.
SVTVFVNNL

SEQ ID NO: 79 - protein, 9 aa, Artificial Sequence
  Amino acid sequence of epitope Peptide (106e) derived from murine cancer cell line.
ASYNGFLPV

SEQ ID NO: 80 - protein, 9 aa, Artificial Sequence
  Amino acid sequence of epitope Peptide (107e) derived from murine cancer cell line.
VLYGLIAAM

SEQ ID NO: 81 - protein, 9 aa, Artificial Sequence
  Amino acid sequence of epitope Peptide (108e) derived from murine cancer cell line.
VSPQHRPVL

SEQ ID NO: 82 - protein, 9 aa, Artificial Sequence
  Amino acid sequence of epitope Peptide (109e) derived from murine cancer cell line.
SAVDFKLHI

SEQ ID NO: 83 - protein, 9 aa, Artificial Sequence
  Amino acid sequence of epitope Peptide (110e) derived from murine cancer cell line.
AMQSRLPTL

SEQ ID NO: 84 - protein, 10 aa, Artificial Sequence
  Amino acid sequence of epitope Peptide (111e) derived from murine cancer cell line.
SAPPLLEGPL

SEQ ID NO: 85 - protein, 9 aa, Artificial Sequence
  Amino acid sequence of epitope Peptide (112e) derived from murine cancer cell line.
VVLDVTASL

SEQ ID NO: 86 - protein, 9 aa, Artificial Sequence
  Amino acid sequence of epitope Peptide (113e) derived from murine cancer cell line.
ASMTNMELM

SEQ ID NO: 87 - protein, 10 aa, Artificial Sequence
  Amino acid sequence of epitope Peptide (114e) derived from murine cancer cell line.
SVLTRLRTPM

SEQ ID NO: 88 - protein, 10 aa, Artificial Sequence
  Amino acid sequence of epitope Peptide (115e) derived from murine cancer cell line.
VSFRSIFKDL

SEQ ID NO: 89 - protein, 9 aa, Artificial Sequence
  Amino acid sequence of epitope Peptide (116e) derived from murine cancer cell line.
SSLTSSVPV

SEQ ID NO: 90 - protein, 9 aa, Artificial Sequence
  Amino acid sequence of epitope Peptide (117e) derived from murine cancer cell line.
VATINFRRL

SEQ ID NO: 91 - protein, 9 aa, Artificial Sequence
  Amino acid sequence of epitope Peptide (118e) derived from murine cancer cell line.
ISFKNLTRV

SEQ ID NO: 92 - protein, 10 aa, Artificial Sequence
  Amino acid sequence of epitope Peptide (119e) derived from murine cancer cell line.
AAMPINKATI

SEQ ID NO: 93 - protein, 9 aa, Artificial Sequence
  Amino acid sequence of epitope Peptide (120e) derived from murine cancer cell line.
CTLQFEAAL

SEQ ID NO: 94 - protein, 9 aa, Artificial Sequence
  Amino acid sequence of epitope Peptide (121e) derived from murine cancer cell line.
VTFFCFQVL

SEQ ID NO: 95 - protein, 9 aa, Artificial Sequence
  Amino acid sequence of epitope Peptide (122e) derived from murine cancer cell line.
MALSTYYAL

SEQ ID NO: 96 - protein, 10 aa, Artificial Sequence
  Amino acid sequence of epitope Peptide (123e) derived from murine cancer cell line.
YSFCDVKQYI

SEQ ID NO: 97 - protein, 9 aa, Artificial Sequence
  Amino acid sequence of epitope Peptide (124e) derived from murine cancer cell line.
KGYPHWPAL

SEQ ID NO: 98 - protein, 9 aa, Artificial Sequence
  Amino acid sequence of epitope Peptide (125e) derived from murine cancer cell line.
AQLQNLTST

SEQ ID NO: 99 - protein, 10 aa, Artificial Sequence
  Amino acid sequence of epitope Peptide (126e) derived from murine cancer cell line.
ASPVSPGEPL

SEQ ID NO: 100 - protein, 9 aa, Artificial Sequence
  Amino acid sequence of epitope Peptide (127e) derived from murine cancer cell line.
RSFTGAVTL

SEQ ID NO: 101 - protein, 9 aa, Artificial Sequence
  Amino acid sequence of epitope Peptide (128e) derived from murine cancer cell line.
RSPTSVNAV

SEQ ID NO: 102 - protein, 9 aa, Artificial Sequence
  Amino acid sequence of epitope Peptide (129e) derived from murine cancer cell line.
VSWNQDPFL

SEQ ID NO: 103 - protein, 9 aa, Artificial Sequence
  Amino acid sequence of epitope Peptide (130e) derived from murine cancer cell line.
WALRIRITL